European Patent Application EP 4 481 038 A1, published December 25, 2024. Title: Novel variant of stress protein and method for preparing L-aromatic amino acid using the same. Applicant: DAESANG CORPORATION. The sequence listing filed with the application follows.

SEQUENCE LISTING (43 sequences)

SEQ ID NO: 1 - protein, 450 aa, synthetic construct
MTKHYDYIAIGGGSGGIASINRAAMYGQKCALIEAKELGGTCVNVGCVPKKVMWHAAQIREAIHMYGPDYGFDITINKFNWETLIASRTAYIDRIHTSYENVLGKNNVDVIKGFARFVDAKTLEVNGETITADHILIATGGRPSHPDIPGVEYGIDSDGFFALPALPERVAVVGAGYIAVELAGVINGLGAKTHLFVRKHAPLRSFDPMISETLVEVMNAEGPQLHTNAIPKAVVKNTDGSLTLELEDGRSETVDCLIWAIGREPANDNINLEAAGVKTNEKGYIVVDKYQNTNIEGIYAVGDNTGAVELTPVAVAAGRRLSERLFNNKPDEHLDYSNIPTVVFSHPPIGTVGLTEPQAREQYGDDQVKVYKSSFTAMYTAVTTHRQPCRMKLVCVGSEEKIVGIHGIGFGMDEMLQGFAVALKMGATKKDFDNTVAIHPTAAEEFVTMR

SEQ ID NO: 2 - DNA, 1353 bp, synthetic construct
  source 1..1353: mol_type = other DNA
atgactaaacactatgattacatcgccatcggcggcggcagcggcggtatcgcctccatcaaccgcgcggctatgtacggccagaaatgtgcgctgattgaagccaaagagctgggcggcacctgcgtaaatgttggctgtgtgccgaaaaaagtgatgtggcacgcggcgcaaatccgtgaagcgatccatatgtacggcccggattatggttttgatatcactatcaataaattcaactgggaaacgttgatcgccagccgtaccgcctatatcgaccgtattcatacttcctatgaaaacgtgctcggtaaaaataacgttgatgtaatcaaaggctttgcccgcttcgttgatgccaaaacgctggaggtaaacggcgaaaccatcacggccgatcatattctgatcgccacaggcggtcgtccgagccacccggatattccgggcgtggaatacggtattgattctgatggcttcttcgcccttcctgctttgccagagcgcgtggcggttgttggcgcgggttacatcgccgttgagctggcgggcgtgattaacggcctcggcgcgaaaacgcatctgtttgtgcgtaaacatgcgccgctgcgcagcttcgacccgatgatttccgaaacgctggtcgaagtgatgaacgccgaaggcccgcagctgcacaccaacgccatcccgaaagcggtagtgaaaaataccgatggtagcctgacgctggagctggaagatggtcgcagtgaaacggtggattgcctgatttgggcgattggtcgcgagcctgccaatgacaacatcaacctggaagccgctggcgttaaaactaacgaaaaaggctatatcgtcgtcgataaatatcaaaacaccaatattgaaggtatttacgcggtgggcgataacacgggtgcagtggagctgacaccggtggcagttgcagcgggtcgccgtctctctgaacgcctgtttaataacaagccggatgagcatctggattacagcaacattccgaccgtggtcttcagccatccgccgattggtactgttggtttaacggaaccgcaggcgcgcgagcagtatggcgacgatcaggtgaaagtgtataaatcctctttcaccgcgatgtataccgccgtcaccactcaccgccagccgtgccgcatgaagctggtgtgcgttggatcggaagagaagattgtcggtattcacggcattggctttggtatggacgaaatgttgcagggcttcgcggtggcgctgaagatgggggcaaccaaaaaagacttcgacaataccgtcgccattcacccaacggcggcagaagagttcgtgacaatgcgttaa

SEQ ID NO: 3 - protein, 450 aa, Escherichia coli
MTKHYDYIAIGGGSGGIASINRAAMYGQKCALIEAKELGGTCVNVGCVPKKVMWHAAQIREAIHMYGPDYGFDTTINKFNWETLIASRTAYIDRIHTSYENVLGKNNVDVIKGFARFVDAKTLEVNGETITADHILIATGGRPSHPDIPGVEYGIDSDGFFALPALPERVAVVGAGYIAVELAGVINGLGAKTHLFVRKHAPLRSFDPMISETLVEVMNAEGPQLHTNAIPKAVVKNTDGSLTLELEDGRSETVDCLIWAIGREPANDNINLEAAGVKTNEKGYIVVDKYQNTNIEGIYAVGDNTGAVELTPVAVAAGRRLSERLFNNKPDEHLDYSNIPTVVFSHPPIGTVGLTEPQAREQYGDDQVKVYKSSFTAMYTAVTTHRQPCRMKLVCVGSEEKIVGIHGIGFGMDEMLQGFAVALKMGATKKDFDNTVAIHPTAAEEFVTMR

SEQ ID NO: 4 - DNA, 1353 bp, Escherichia coli
  source 1..1353: mol_type = genomic DNA
atgactaaacactatgattacatcgccatcggcggcggcagcggcggtatcgcctccatcaaccgcgcggctatgtacggccagaaatgtgcgctgattgaagccaaagagctgggcggcacctgcgtaaatgttggctgtgtgccgaaaaaagtgatgtggcacgcggcgcaaatccgtgaagcgatccatatgtacggcccggattatggttttgataccactatcaataaattcaactgggaaacgttgatcgccagccgtaccgcctatatcgaccgtattcatacttcctatgaaaacgtgctcggtaaaaataacgttgatgtaatcaaaggctttgcccgcttcgttgatgccaaaacgctggaggtaaacggcgaaaccatcacggccgatcatattctgatcgccacaggcggtcgtccgagccacccggatattccgggcgtggaatacggtattgattctgatggcttcttcgcccttcctgctttgccagagcgcgtggcggttgttggcgcgggttacatcgccgttgagctggcgggcgtgattaacggcctcggcgcgaaaacgcatctgtttgtgcgtaaacatgcgccgctgcgcagcttcgacccgatgatttccgaaacgctggtcgaagtgatgaacgccgaaggcccgcagctgcacaccaacgccatcccgaaagcggtagtgaaaaataccgatggtagcctgacgctggagctggaagatggtcgcagtgaaacggtggattgcctgatttgggcgattggtcgcgagcctgccaatgacaacatcaacctggaagccgctggcgttaaaactaacgaaaaaggctatatcgtcgtcgataaatatcaaaacaccaatattgaaggtatttacgcggtgggcgataacacgggtgcagtggagctgacaccggtggcagttgcagcgggtcgccgtctctctgaacgcctgtttaataacaagccggatgagcatctggattacagcaacattccgaccgtggtcttcagccatccgccgattggtactgttggtttaacggaaccgcaggcgcgcgagcagtatggcgacgatcaggtgaaagtgtataaatcctctttcaccgcgatgtataccgccgtcaccactcaccgccagccgtgccgcatgaagctggtgtgcgttggatcggaagagaagattgtcggtattcacggcattggctttggtatggacgaaatgttgcagggcttcgcggtggcgctgaagatgggggcaaccaaaaaagacttcgacaataccgtcgccattcacccaacggcggcagaagagttcgtgacaatgcgttaa

SEQ ID NO: 5 - protein, 41 aa, synthetic construct
MISTVALFWALCVVCIVNMARYFSSLRALLVVLRNCDPLLY

SEQ ID NO: 6 - DNA, 336 bp, synthetic construct
  source 1..336: mol_type = other DNA
atgataagcaccgtcgcattattttgggctttatgtgtcgtttgcattgttaacatggcgcgctatttctcatcactacgcgcgttgttagtggtactgcgtaactgcgatccattgctctattaatatgttgatggagggggcttttttacctcacatggccaacccaacaaacaggtgcgtctcgtttggtatatctatgcccaacgttatcgcgatcatcacgatgatgaatttattcgccgctgtgagcgggtgcgtcggcagtttattctgaccagcgcattgtgtggtctggtggtggtcagcctgattgcattgatgatttggcattaa

SEQ ID NO: 7 - protein, 111 aa, Escherichia coli
MISTVALFWALCVVCIVNMARYFSSLRALLVVLRNCDPLLYQYVDGGGFFTSHGQPNKQVRLVWYIYAQRYRDHHDDEFIRRCERVRRQFILTSALCGLVVVSLIALMIWH

SEQ ID NO: 8 - DNA, 336 bp, Escherichia coli
  source 1..336: mol_type = genomic DNA
atgataagcaccgtcgcattattttgggctttatgtgtcgtttgcattgttaacatggcgcgctatttctcatcactacgcgcgttgttagtggtactgcgtaactgcgatccattgctctatcaatatgttgatggagggggcttttttacctcacatggccaacccaacaaacaggtgcgtctcgtttggtatatctatgcccaacgttatcgcgatcatcacgatgatgaatttattcgccgctgtgagcgggtgcgtcggcagtttattctgaccagcgcattgtgtggtctggtggtggtcagcctgattgcattgatgatttggcattaa

SEQ ID NO: 9 - DNA, 30 bp, synthetic construct
  source 1..30: mol_type = other DNA
caattttattatagtaattgactattatac

SEQ ID NO: 10 - DNA, 40 bp, synthetic construct
  source 1..40: mol_type = other DNA
ttgataccaccaattttattatagtaattgactattatac

SEQ ID NO: 11 - DNA, 40 bp, synthetic construct
  source 1..40: mol_type = other DNA
gtggtatcaaaaccataatcgttttagagctagaaatagc

SEQ ID NO: 12 - DNA, 30 bp, synthetic construct
  source 1..30: mol_type = other DNA
aaccataatcgttttagagctagaaatagc

SEQ ID NO: 13 - DNA, 21 bp, synthetic construct
  source 1..21: mol_type = other DNA
gagcctgtcggcctacctgct

SEQ ID NO: 14 - DNA, 20 bp, synthetic construct
  source 1..20: mol_type = other DNA
cggccggcatgagcctgtcg

SEQ ID NO: 15 - DNA, 30 bp, synthetic construct
  source 1..30: mol_type = other DNA
atgccggccgaataacgtgctgccgtggct

SEQ ID NO: 16 - DNA, 20 bp, synthetic construct
  source 1..20: mol_type = other DNA
aataacgtgctgccgtggct

SEQ ID NO: 17 - DNA, 20 bp, synthetic construct
  source 1..20: mol_type = other DNA
ataatccgggccgtacatat

SEQ ID NO: 18 - DNA, 20 bp, synthetic construct
  source 1..20: mol_type = other DNA
tatcaaaaccataatccggg

SEQ ID NO: 19 - DNA, 35 bp, synthetic construct
  source 1..35: mol_type = other DNA
ggttttgatatcactatcaataaattcaactggga

SEQ ID NO: 20 - DNA, 25 bp, synthetic construct
  source 1..25: mol_type = other DNA
tcactatcaataaattcaactggga

SEQ ID NO: 21 - DNA, 25 bp, synthetic construct
  source 1..25: mol_type = other DNA
gcgttttcgcgccgaggccgttaat

SEQ ID NO: 22 - DNA, 20 bp, synthetic construct
  source 1..20: mol_type = other DNA
acaaacagatgcgttttcgc

SEQ ID NO: 23 - DNA, 33 bp, synthetic construct
  source 1..33: mol_type = other DNA
atctgtttgtgagctcctgaaaatctcgataac

SEQ ID NO: 24 - DNA, 23 bp, synthetic construct
  source 1..23: mol_type = other DNA
gagctcctgaaaatctcgataac

SEQ ID NO: 25 - DNA, 20 bp, synthetic construct
  source 1..20: mol_type = other DNA
tctggaagcgaccggtattc

SEQ ID NO: 26 - DNA, 20 bp, synthetic construct
  source 1..20: mol_type = other DNA
ctgcgaccatcttccagctc

SEQ ID NO: 27 - DNA, 40 bp, synthetic construct
  source 1..40: mol_type = other DNA
gatagagcaacaattttattatagtaattgactattatac

SEQ ID NO: 28 - DNA, 40 bp, synthetic construct
  source 1..40: mol_type = other DNA
ttgctctatcaatatgttgagttttagagctagaaatagc

SEQ ID NO: 29 - DNA, 30 bp, synthetic construct
  source 1..30: mol_type = other DNA
aatatgttgagttttagagctagaaatagc

SEQ ID NO: 30 - DNA, 30 bp, synthetic construct
  source 1..30: mol_type = other DNA
atgccggccgatagtggttaaccttctgga

SEQ ID NO: 31 - DNA, 20 bp, synthetic construct
  source 1..20: mol_type = other DNA
atagtggttaaccttctgga

SEQ ID NO: 32 - DNA, 20 bp, synthetic construct
  source 1..20: mol_type = other DNA
ggatcgcagttacgcagtac

SEQ ID NO: 33 - DNA, 20 bp, synthetic construct
  source 1..20: mol_type = other DNA
atagagcaatggatcgcagt

SEQ ID NO: 34 - DNA, 30 bp, synthetic construct
  source 1..30: mol_type = other DNA
attgctctattaatatgttgatggaggggg

SEQ ID NO: 35 - DNA, 20 bp, synthetic construct
  source 1..20: mol_type = other DNA
taatatgttgatggaggggg

SEQ ID NO: 36 - DNA, 24 bp, synthetic construct
  source 1..24: mol_type = other DNA
attttgcgtttgtaatcagtctcg

SEQ ID NO: 37 - DNA, 20 bp, synthetic construct
  source 1..20: mol_type = other DNA
gcatcaggcaattttgcgtt

SEQ ID NO: 38 - DNA, 33 bp, synthetic construct
  source 1..33: mol_type = other DNA
tgcctgatgcgagctcctgaaaatctcgataac

SEQ ID NO: 39 - DNA, 23 bp, synthetic construct
  source 1..23: mol_type = other DNA
gagctcctgaaaatctcgataac

SEQ ID NO: 40 - DNA, 20 bp, synthetic construct
  source 1..20: mol_type = other DNA
agcgtttcttgtgccgttac

SEQ ID NO: 41 - DNA, 20 bp, synthetic construct
  source 1..20: mol_type = other DNA
gattgtgacatagtgcgctt

SEQ ID NO: 42 - DNA, 3234 bp, synthetic construct
  source 1..3234: mol_type = other DNA
tttccataggctccgcccccctgacgagcatcacaaaaatcgacgctcaagtcagaggtggcgaaacccgacaggactataaagataccaggcgtttccccctggaagctccctcgtgcgctctcctgttccgaccctgccgcttaccggatacctgtccgcctttctcccttcgggaagcgtggcgctttctcatagctcacgctgtaggtatctcagttcggtgtaggtcgttcgctccaagctgggctgtgtgcacgaaccccccgttcagcccgaccgctgcgccttatccggtaactatcgtcttgagtccaacccggtaagacacgacttatcgccactggcagcagccactggtaacaggattagcagagcgaggtatgtaggcggtgctacagagttcttgaagtggtggcctaactacggctacactagaaggacagtatttggtatctgcgctctgctgaagccagttaccttcggaaaaagagttggtagctcttgatccggcaaacaaaccaccgctggtagcggtggtttttttgtttgcaagcagcagattacgcgcagaaaaaaaggatctcaagaagatcctttgatcttttctacggggtctgacgctcagtggaacgaaaactcacgttaagggattttggtcatgagattatcaaaaaggatcttcacctagatccttttaaattaaaaatgaagttttaaatcaatctaaagtatatatgagtaaacttggtctgacagttaaaagattgacagtataatagtcaattactataataaaattgatgcgcaggtgaaacacctgctgcagttttagagctagaaatagcaagttaaaataaggctagtccgttatcaacttgaaaaagtggcaccgagtcggtgctttttttcgttttccgggacgccctcgcggacgtgctcatagtccacgacgcccgtgattttgtagccctggccgacggccagcaggtaggccgacaggctcatgccggccggagctcctgaaaatctcgataactcaaaaaatacgcccggtagtgatcttatttcattatggtgaaagttggaacctcttaggatcctctagatttaagaaggagatatacataaaactccttctgagctagttctctagcattctattattttgattcgacaccttaataatagcagaaggagtttttacctgtcaaagaaccatcaaacccttgatacacaaggctttgacctaattttgaaaaatgatgttgtttctatatagtatcaagataagaaagaaaaggatttttcgctacgctcaaatcctttcccgtcacgggcttctcagggcgttttatggcgggtctgctatgtggtgctatctgactttttgctgttcagcagttcctgccctctgattttccagtctgaccacttcggattatcccgtgacaggtcattcagactggctaatgcacccagtaaggcagcggtatcatcaacggggtctgacgctcagtggaacgaaaactcacgttaagggattttggtcatgagattatcaaaaaggatcttcacctagatccttttaaattaaaaatgaagttttaaatcaatctaaagtatatatgagtaaacttggtctgacagttaccaatgcttaatcagtgaggcacctatctcagcgatctgtctatttcgttcatccatagttgcctgactccccgtcgtgtagataactacgatacgggagggcttaccatctggccccagtgctgcaatgataccgcgagacccacgctcaccggctccagatttatcagcaataaaccagccagccggaagggccgagcgcagaagtggtcctgcaactttatccgcctccatccagtctattaattgttgccgggaagctagagtaagtagttcgccagttaatagtttgcgcaacgttgttgccattgctacaggcatcgtggtgtcacgctcgtcgtttggtatggcttcattcagctccggttcccaacgatcaaggcgagttacatgatcccccatgttgtgcaaaaaagcggttagctccttcggtcctccgatcgttgtcagaagtaagttggccgcagtgttatcactcatggttatggcagcactgcataattctcttactgtcatgccatccgtaagatgcttttctgtgactggtgagtactcaaccaagtcattctgagaatagtgtatgcggcgaccgagttgctcttgcccggcgtcaatacgggataataccgcgccacatagcagaactttaaaagtgctcatcattggaaaacgttcttcggggcgaaaactctcaaggatcttaccgctgttgagatccagttcgatgtaacccactcgtgcacccaactgatcttcagcatcttttactttcaccagcgtttctgggtgagcaaaaacaggaaggcaaaatgccgcaaaaaagggaataagggcgacacggaaatgttgaatactcatactcttcctttttcaatattattgaagcatttatcagggttattgtctcatgagcggatacatatttgaatgtatttagaaaaataaacaaataggggttccgcgcacatttccccgaaaagtgccaccaaaaaaacacaaaagaccacattttttaatgtggtctttattcttcaactaaagcacccattagttcaacaaacgaaaattggataaagtgggatatttttaaaatatatatttatgttacagtaagctgcctcgcgcgtttcggtgatgacggtgaaaacctctgacacatgcagctcccggagacggtcacagcttgtctgtaagcggatgccgggagcagacaagcccgtcagggcgcgtcagcgggtgttggcgggtgtcggggcgcagccatgacccagtcacgtagcgatagcggagtgtatactggcttaactatgcggcatcagagcagattgtactgagagtgcaccatatgcggtgtgaaataccgcacagatgcgtaaggagaaaataccgcatcaggcgctcttccgcttcctcgctcactgactcgctgcgctcggtcgttcggctgcggcgagcggtatcagctcactcaaaggcggtaatacggttatccacagaatcaggggataacgcaggaaagaacatgtgagcaaaaggccagcaaaaggccaggaaccgtaaaaaggccgcgttgctggcgtt

SEQ ID NO: 43 - DNA, 9656 bp, synthetic construct
  source 1..9656: mol_type = other DNA
aaagccatgacaaaaacgcgtaacaaaagtgtctataatcacggcagaaaagtccacattgattatttgcacggcgtcacactttgctatgccatagcatttttatccataagattagcggatcctacctgacgctttttatcgcaactctctactgtttctccatacccgtttttttgggaattcgagctctaaggaggttataaaaaatggatattaatactgaaactgagatcaagcaaaagcattcactaaccccctttcctgttttcctaatcagcccggcatttcgcgggcgatattttcacagctatttcaggagttcagccatgaacgcttattacattcaggatcgtcttgaggctcagagctgggcgcgtcactaccagcagctcgcccgtgaagagaaagaggcagaactggcagacgacatggaaaaaggcctgccccagcacctgtttgaatcgctatgcatcgatcatttgcaacgccacggggccagcaaaaaatccattacccgtgcgtttgatgacgatgttgagtttcaggagcgcatggcagaacacatccggtacatggttgaaaccattgctcaccaccaggttgatattgattcagaggtataaaacgaatgagtactgcactcgcaacgctggctgggaagctggctgaacgtgtcggcatggattctgtcgacccacaggaactgatcaccactcttcgccagacggcatttaaaggtgatgccagcgatgcgcagttcatcgcattactgatcgttgccaaccagtacggccttaatccgtggacgaaagaaatttacgcctttcctgataagcagaatggcatcgttccggtggtgggcgttgatggctggtcccgcatcatcaatgaaaaccagcagtttgatggcatggactttgagcaggacaatgaatcctgtacatgccggatttaccgcaaggaccgtaatcatccgatctgcgttaccgaatggatggatgaatgccgccgcgaaccattcaaaactcgcgaaggcagagaaatcacggggccgtggcagtcgcatcccaaacggatgttacgtcataaagccatgattcagtgtgcccgtctggccttcggatttgctggtatctatgacaaggatgaagccgagcgcattgtcgaaaatactgcatacactgcagaacgtcagccggaacgcgacatcactccggttaacgatgaaaccatgcaggagattaacactctgctgatcgccctggataaaacatgggatgacgacttattgccgctctgttcccagatatttcgccgcgacattcgtgcatcgtcagaactgacacaggccgaagcagtaaaagctcttggattcctgaaacagaaagccgcagagcagaaggtggcagcatgacaccggacattatcctgcagcgtaccgggatcgatgtgagagctgtcgaacagggggatgatgcgtggcacaaattacggctcggcgtcatcaccgcttcagaagttcacaacgtgatagcaaaaccccgctccggaaagaagtggcctgacatgaaaatgtcctacttccacaccctgcttgctgaggtttgcaccggtgtggctccggaagttaacgctaaagcactggcctggggaaaacagtacgagaacgacgccagaaccctgtttgaattcacttccggcgtgaatgttactgaatccccgatcatctatcgcgacgaaagtatgcgtaccgcctgctctcccgatggtttatgcagtgacggcaacggccttgaactgaaatgcccgtttacctcccgggatttcatgaagttccggctcggtggtttcgaggccataaagtcagcttacatggcccaggtgcagtacagcatgtgggtgacgcgaaaaaatgcctggtactttgccaactatgacccgcgtatgaagcgtgaaggcctgcattatgtcgtgattgagcgggatgaaaagtacatggcgagttttgacgagatcgtgccggagttcatcgaaaaaatggacgaggcactggctgaaattggttttgtatttggggagcaatggcgatgagatctaaagaggagaaaggatctatggataagaaatactcaataggcttagatatcggcacaaatagcgtcggatgggcggtgatcactgatgaatataaggttccgtctaaaaagttcaaggttctgggaaatacagaccgccacagtatcaaaaaaaatcttataggggctcttttatttgacagtggagagacagcggaagcgactcgtctcaaacggacagctcgtagaaggtatacacgtcggaagaatcgtatttgttatctacaggagattttttcaaatgagatggcgaaagtagatgatagtttctttcatcgacttgaagagtcttttttggtggaagaagacaagaagcatgaacgtcatcctatttttggaaatatagtagatgaagttgcttatcatgagaaatatccaactatctatcatctgcgaaaaaaattggtagattctactgataaagcggatttgcgcttaatctatttggccttagcgcatatgattaagtttcgtggtcattttttgattgagggagatttaaatcctgataatagtgatgtggacaaactatttatccagttggtacaaacctacaatcaattatttgaagaaaaccctattaacgcaagtggagtagatgctaaagcgattctttctgcacgattgagtaaatcaagacgattagaaaatctcattgctcagctccccggtgagaagaaaaatggcttatttgggaatctcattgctttgtcattgggtttgacccctaattttaaatcaaattttgatttggcagaagatgctaaattacagctttcaaaagatacttacgatgatgatttagataatttattggcgcaaattggagatcaatatgctgatttgtttttggcagctaagaatttatcagatgctattttactttcagatatcctaagagtaaatactgaaataactaaggctcccctatcagcttcaatgattaaacgctacgatgaacatcatcaagacttgactcttttaaaagctttagttcgacaacaacttccagaaaagtataaagaaatcttttttgatcaatcaaaaaacggatatgcaggttatattgatgggggagctagccaagaagaattttataaatttatcaaaccaattttagaaaaaatggatggtactgaggaattattggtgaaactaaatcgtgaagatttgctgcgcaagcaacggacctttgacaacggctctattccccatcaaattcacttgggtgagctgcatgctattttgagaagacaagaagacttttatccatttttaaaagacaatcgtgagaagattgaaaaaatcttgacttttcgaattccttattatgttggtccattggcgcgtggcaatagtcgttttgcatggatgactcggaagtctgaagaaacaattaccccatggaattttgaagaagttgtcgataaaggtgcttcagctcaatcatttattgaacgcatgacaaactttgataaaaatcttccaaatgaaaaagtactaccaaaacatagtttgctttatgagtattttacggtttataacgaattgacaaaggtcaaatatgttactgaaggaatgcgaaaaccagcatttctttcaggtgaacagaagaaagccattgttgatttactcttcaaaacaaatcgaaaagtaaccgttaagcaattaaaagaagattatttcaaaaaaatagaatgttttgatagtgttgaaatttcaggagttgaagatagatttaatgcttcattaggtacctaccatgatttgctaaaaattattaaagataaagattttttggataatgaagaaaatgaagatatcttagaggatattgttttaacattgaccttatttgaagatagggagatgattgaggaaagacttaaaacatatgctcacctctttgatgataaggtgatgaaacagcttaaacgtcgccgttatactggttggggacgtttgtctcgaaaattgattaatggtattagggataagcaatctggcaaaacaatattagattttttgaaatcagatggttttgccaatcgcaattttatgcagctgatccatgatgatagtttgacatttaaagaagacattcaaaaagcacaagtgtctggacaaggcgatagtttacatgaacatattgcaaatttagctggtagccctgctattaaaaaaggtattttacagactgtaaaagttgttgatgaattggtcaaagtaatggggcggcataagccagaaaatatcgttattgaaatggcacgtgaaaatcagacaactcaaaagggccagaaaaattcgcgagagcgtatgaaacgaatcgaagaaggtatcaaagaattaggaagtcagattcttaaagagcatcctgttgaaaatactcaattgcaaaatgaaaagctctatctctattatctccaaaatggaagagacatgtatgtggaccaagaattagatattaatcgtttaagtgattatgatgtcgatcacattgttccacaaagtttccttaaagacgattcaatagacaataaggtcttaacgcgttctgataaaaatcgtggtaaatcggataacgttccaagtgaagaagtagtcaaaaagatgaaaaactattggagacaacttctaaacgccaagttaatcactcaacgtaagtttgataatttaacgaaagctgaacgtggaggtttgagtgaacttgataaagctggttttatcaaacgccaattggttgaaactcgccaaatcactaagcatgtggcacaaattttggatagtcgcatgaatactaaatacgatgaaaatgataaacttattcgagaggttaaagtgattaccttaaaatctaaattagtttctgacttccgaaaagatttccaattctataaagtacgtgagattaacaattaccatcatgcccatgatgcgtatctaaatgccgtcgttggaactgctttgattaagaaatatccaaaacttgaatcggagtttgtctatggtgattataaagtttatgatgttcgtaaaatgattgctaagtctgagcaagaaataggcaaagcaaccgcaaaatatttcttttactctaatatcatgaacttcttcaaaacagaaattacacttgcaaatggagagattcgcaaacgccctctaatcgaaactaatggggaaactggagaaattgtctgggataaagggcgagattttgccacagtgcgcaaagtattgtccatgccccaagtcaatattgtcaagaaaacagaagtacagacaggcggattctccaaggagtcaattttaccaaaaagaaattcggacaagcttattgctcgtaaaaaagactgggatccaaaaaaatatggtggttttgatagtccaacggtagcttattcagtcctagtggttgctaaggtggaaaaagggaaatcgaagaagttaaaatccgttaaagagttactagggatcacaattatggaaagaagttcctttgaaaaaaatccgattgactttttagaagctaaaggatataaggaagttaaaaaagacttaatcattaaactacctaaatatagtctttttgagttagaaaacggtcgtaaacggatgctggctagtgccggagaattacaaaaaggaaatgagctggctctgccaagcaaatatgtgaattttttatatttagctagtcattatgaaaagttgaagggtagtccagaagataacgaacaaaaacaattgtttgtggagcagcataagcattatttagatgagattattgagcaaatcagtgaattttctaagcgtgttattttagcagatgccaatttagataaagttcttagtgcatataacaaacatagagacaaaccaatacgtgaacaagcagaaaatattattcatttatttacgttgacgaatcttggagctcccgctgcttttaaatattttgatacaacaattgatcgtaaacgatatacgtctacaaaagaagttttagatgccactcttatccatcaatccatcactggtctttatgaaacacgcattgatttgagtcagctaggaggtgactaacgcatcctcacgataatatccgggtaggcgcaatcactttcgtctactccgttacaaagcgaggctgggtatttcccggcctttctgttatccgaaatccactgaaagcacagcggctggctgaggagataaataataaacgaggggctgtatgcacaaagcatcttctgttgagttaagaacgagtatcgagatggcacatagccttgctcaaattggaatcaggtttgtgccaataccagtagaaacagacgaagaatccatgggtatggacagttttccctttgatatgtaacggtgaacagttgttctacttttgtttgttagtcttgatgcttcactgatagatacaagagccaaatctagtaatattttatctgattaataagatgatcttcttgagatcgttttggtctgcgcgtaatctcttgctctgaaaacgaaaaaaccgccttgcagggcggtttttcgaaggttctctgagctaccaactctttgaaccgaggtaactggcttggaggagcgcagtcaccaaaacttgtcctttcagtttagccttaaccggcgcatgacttcaagactaactcctctaaatcaattaccagtggctgctgccagtggtgcttttgcatgtctttccgggttggactcaagacgatagttaccggataaggcgcagcggtcggactgaacggggggttcgtgcatacagtccagcttggagcgaactgcctacccggaactgagtgtcaggcgtggaatgagacaaacgcggccataacagcggaatgacaccggtaaaccgaaaggcaggaacaggagagcgcacgagggagccgccagggggaaacgcctggtatctttatagtcctgtcgggtttcgccaccactgatttgagcgtcagatttcgtgatgcttgtcaggggggcggagcctatggaaaaacggctttgccgcggccccgctgaatattccttttgtctccgaccatcaggcacctgagtcgctgtctttttcgtgacattcagttcgctgcgctcacggctctggcagtgaatgggggtaaatggcactacaggcgccttttatggattcatgcaaggaaactacccataatacaagaaaagatgtggtctttattcttcaactaaagcacccattagttcaacaaacgaaaattggataaagtgggatatttttaaaatatatatttatgttacctggcagagcctgtactttttacagtcggttttctaatgtcactaacctgccccgttagtcgccatttgcatcgatttattatgacaacttgacggctacatcattcactttttcttcacaaccggcacggaactcgctcgggctggccccggtgcattttttaaatacccgcgagaaatagagttgatcgtcaaaaccaacattgcgaccgacggtggcgataggcatccgggtggtgctcaaaagcagcttcgcctggctgatacgttggtcctcgcgccagcttaagacgctaatccctaactgctggcggaaaagatgtgacagacgcgacggcgacaagcaaacatgctgtgcgacgctggcgatatcaaaattgctgtctgccaggtgatcgctgatgtactgacaagcctcgcgtacccgattatccatcggtggatggagcgactcgttaatcgcttccatgcgccgcagtaacaattgctcaagcagatttatcgccagcagctccgaatagcgcccttccccttgcccggcgttaatgatttgcccaaacaggtcgctgaaatgcggctggtgcgcttcatccgggcgaaagaaccccgtattggcaaatattgacggccagttaagccattcatgccagtaggcgcgcggacgaaagtaaacccactggtgataccattcgcgagcctccggatgacgaccgtagtgatgaatctctcctggcgggaacagcaaaatatcacccggtcggcaaacaaattctcgtccctgatttttcaccaccccctgaccgcgaatggtgagattgagaatataacctttcattcccagcggtcggtcgataaaaaaatcgagataaccgttggcctcaatcggcgttaaacccgccaccagatgggcattaaacgagtatcccggcagcaggggatcattttgcgcttcagccatacttttcatactcccgccattcagagaagaaaccaattgtccatattgcatcagacattgccgtcactgcgtcttttactggctcttctcgctaaccaaaccggtaaccccgcttattaaaagcattctgtaacaaagcgggaccagtaatagaaagtgagggagccacggttgatgagagctttgttgtaggtggaccagttggtgattttgaacttttgctttgccacggaacggtctgcgttgtcgggaagatgcgtgatctgatccttcaactcagcaaaagttcgatttattcaacaaagccacgttgtgtctcaaaatctctgatgttacattgcacaagataaaaatatatcatcatgaacaataaaactgtctgcttacataaacagtaatacaaggggtgttatgagccatattcaacgggaaacgtcttgctcgaggccgcgattaaattccaacatggatgctgatttatatgggtataaatgggctcgcgataatgtcgggcaatcaggtgcgacaatctatcgattgtatgggaagcccgatgcgccagagttgtttctgaaacatggcaaaggtagcgttgccaatgatgttacagatgagatggtcagactaaactggctgacggaatttatgcctcttccgaccatcaagcattttatccgtactcctgatgatgcatggttactcaccactgcgatccccgggaaaacagcattccaggtattagaagaatatcctgattcaggtgaaaatattgttgatgcgctggcagtgttcctgcgccggttgcattcgattcctgtttgtaattgtccttttaacagcgatcgcgtatttcgtctcgctcaggcgcaatcacgaatgaataacggtttggttgatgcgagtgattttgatgacgagcgtaatggctggcctgttgaacaagtctggaaagaaatgcataagcttttgccattctcaccggattcagtcgtcactcatggtgatttctcacttgataaccttatttttgacgaggggaaattaataggttgtattgatgttggacgagtcggaatcgcagaccgataccaggatcttgccatcctatggaactgcctcggtgagttttctccttcattacagaaacggctttttcaaaaatatggtattgataatcctgatatgaataaattgcagtttcatttgatgctcgatgagtttttctaatcagaattggttaattggttgtaaca